European Patent Specification EP 3 795 588 B1, published December 18, 2024. Title: HLA-B57 open conformers. Applicant: Universitaet Zuerich Universitaet Basel. The sequence listing filed with the application follows.

SEQUENCE LISTING (110 sequences)

SEQ ID NO: 1 - protein, 362 aa, Homo sapiens [sequence omitted]

SEQ ID NO: 2 - protein, 181 aa, Homo sapiens
SHSMRYFYTAMSRPGRGEPRFIAVGYVDDTQFVRFDSDAASPRMAPRAPWIEQEGPEYWDGETRNMKASAQTYRENLRIALRYYNQSEAGSHIIQVMYGCDVGPDGRLLRGHDQSAYDGKDYIALNEDLSSWTAADTAAQITQRKWEAARVAEQLRAYLEGLCVEWLRRYLENGKETLQRA

SEQ ID NO: 3 - protein, 181 aa, Homo sapiens; identical to SEQ ID NO: 2

SEQ ID NO: 4 - protein, 181 aa, Homo sapiens; identical to SEQ ID NO: 2

SEQ ID NO: 5 - protein, 181 aa, Homo sapiens; identical to SEQ ID NO: 2

SEQ ID NO: 6 - protein, 181 aa, Homo sapiens; identical to SEQ ID NO: 2

SEQ ID NO: 7 - protein, 273 aa, Homo sapiens
SHSMRYFYTAMSRPGRGEPRFIAVGYVDDTQFVRFDSDAASPRMAPRAPWIEQEGPEYWDGETRNMKASAQTYRENLRIALRYYNQSEAGSHIIQVMYGCDVGPDGRLLRGHDQSAYDGKDYIALNEDLSSWTAADTAAQITQRKWEAARVAEQLRAYLEGLCVEWLRRYLENGKETLQRADPPKTHVTHHPISDHEATLRCWALGFYPAEITLTWQRDGEDQTQDTELVETRPAGDRTFQKWAAVVVPSGEEQRYTCHVQHEGLPKPLTLRW

SEQ ID NO: 8 - protein, 181 aa, Homo sapiens; identical to SEQ ID NO: 2

SEQ ID NO: 9 - protein, 181 aa, Homo sapiens; identical to SEQ ID NO: 2

SEQ ID NO: 10 - protein, 181 aa, Homo sapiens; identical to SEQ ID NO: 2

SEQ ID NO: 11 - protein, 273 aa, Homo sapiens; identical to SEQ ID NO: 7

SEQ ID NO: 12 - protein, 181 aa, Homo sapiens; identical to SEQ ID NO: 2

SEQ ID NO: 13 - protein, 362 aa, Homo sapiens [sequence omitted]

SEQ ID NO: 14 - protein, 181 aa, Homo sapiens; identical to SEQ ID NO: 2

SEQ ID NO: 15 - protein, 181 aa, Homo sapiens; identical to SEQ ID NO: 2

SEQ ID NO: 16 - protein, 181 aa, Homo sapiens; identical to SEQ ID NO: 2

SEQ ID NO: 17 - protein, 337 aa, Homo sapiens
MRVTAPRTVLLLLWGAVALTETWAGSHSMRYFYTAMSRPGRGEPRFIAVGYVDDTQFVRFDSDAASPRMAPRAPWIEQEGPEYWDGETRNMKASAQTYRENLRIALRYYNQSEAGSHIIQVMYGCDVGPDGRLLRGHDQSAYDGKDYIALNEDLSSWTAADTAAQITQRKWEAARVAEQLRAYLEGLCVEWLRRYLENGKETLQRADPPKTHVTHHPISDHEATLRCWALGFYPAEITLTWQRDGEDQTQDTELVETRPAGDRTFQKWAAVVVPSGEEQRYTCHVQHEGLPKPLTLRWEPSSQSTVPIVGIVAGLAVLAVVVIGAVVAAVMCRRKSS

SEQ ID NO: 18 - protein, 181 aa, Homo sapiens; identical to SEQ ID NO: 2

SEQ ID NO: 19 - protein, 298 aa, Homo sapiens
MRVTAPRTVLLLLWGAVALTETWAGSHSMRYFYTAMSRPGRGEPRFIAVGYVDDTQFVRFDSDAASPRMAPRAPWIEQEGPEYWDGETRNMKASAQTYRENLRIALRYYNQSEAGSHIIQVMYGCDVGPDGRLLRGHDQSAYDGKDYIALNEDLSSWTAADTAAQITQRKWEAARVAEQLRAYLEGLCVEWLRRYLENGKETLQRADPPKTHVTHHPISDHEATLRCWALGFYPAEITLTWQRDGEDQTQDTELVETRPAGDRTFQKWAAVVVPSGEEQRYTCHVQHEGLPKPLTLRW

SEQ ID NO: 20 - protein, 181 aa, Homo sapiens; identical to SEQ ID NO: 2

SEQ ID NO: 21 - protein, 273 aa, Homo sapiens; identical to SEQ ID NO: 7

SEQ ID NO: 22 - protein, 181 aa, Homo sapiens; identical to SEQ ID NO: 2

SEQ ID NO: 23 - protein, 362 aa, Homo sapiens [sequence omitted]

SEQ ID NO: 24 - protein, 181 aa, Homo sapiens
SHSMRYFYTAMSRPGRGEPRFIAVGYVDDTQFVRFDSDAASPRMAPRAPWIEQEGPEYWDGETRNMKASAQTYRENLRIALRYYNQSEAGSHIIQVMYGCDVGPDGRLLRGHNQYAYDGKDYIALNEDLSSWTAADTAAQITQRKWEAARVAEQRRAYLEGLCVEWLRRYLENGKETLQRA

SEQ ID NO: 25 - protein, 362 aa, Homo sapiens [sequence omitted]

SEQ ID NO: 26 - protein, 273 aa, Homo sapiens
SHSMRYFYTAMSRPGRGEPRFIAVGYVDDTQFVRFDSDAASPRMAPRAPWIEQEGPEYWDGETRNMKASAQTYRENLRIALRYYNQSEAGSHIIQVMYGCDVGPDGRLLRGHNQYAYDGKDYIALNEDLSSWTAADTAAQITQRKWEAARVAEQLRAYLEGLCVEWLRRYLENGKETLQRADPPKTHVTHHPISDHEATLRCWALGFYPAEITLTWQRDGEDQTQDTELVETRPAGDRTFQKWAAVVVPSGEEQRYTCHVQHEGLPKPLTLRW

SEQ ID NO: 27 - protein, 273 aa, Homo sapiens
SHSMRYFYTAMSRPGRGEPRFIAVGYVDDTQFVRFDSDAASPRMAPRAPWIEQEGPEYWDGETRNMKASAQTYRENLRIALRYYNQSEAGSHIIQVMYGCDVGPDGRLLRGYDQDAYDGKDYIALNEDLSSWTAADTAAQITQRKWEAARVAEQRRAYLEGLCVEWLRRYLENGKETLQRADPPKTHVTHHPISDHEATLRCWALGFYPAEITLTWQRDGEDQTQDTELVETRPAGDRTFQKWAAVVVPSGEEQRYTCHVQHEGLPKPLTLRW

SEQ ID NO: 28 - protein, 181 aa, Homo sapiens
SHSMRYFYTAMSRPGRGEPRFIAVGYVDDTQFVRFDSDAASPRMAPRAPWIEQEGPEYWDGETRNMKASAQTYRENLRIALRYYNQSEAGSHIIQVMYGCDVGPDGRLLRGYDQDAYDGKDYIALNEDLSSWTAADTAAQITQRKWEAARVAEQRRAYLEGLCVEWLRRYLENGKETLQRA

SEQ ID NO: 29 - protein, 362 aa, Homo sapiens [sequence omitted]

SEQ ID NO: 30 - protein, 362 aa, Homo sapiens [sequence omitted]

SEQ ID NO: 31 - protein, 181 aa, Homo sapiens
SHSMRYFYTAMSRPGRGEPRFIAVGYVDDTQFVRFDSDAASPRMAPRAPWIEQEGPEYWDGETRNMKASAQTYRENLRIALRYYNQSEAGSHIIQVMYGCDVGPDGRLLRGHNQYAYDGKDYIALNEDLSSWTAADTAAQITQRKWEAARVAEQLRAYLEGLCVESLRRYLENGKETLQRA

SEQ ID NO: 32 - protein, 181 aa, Homo sapiens
SHSMRYFYTAMSRPGRGEPRFIAVGYVDDTQFVRFDSDAASPRMAPRAPWIEQEGPEYWDGETRNMKASAQTYRENLRIALPYYNQSEAGSHIIQVMYGCDVGPDGRLLRGHDQSAYDGKDYIALNEDLSSWTAADTAAQITQRKWEAARVAEQLRAYLEGLCVEWLRRYLENGKETLQRA

SEQ ID NO: 33 - protein, 181 aa, Homo sapiens
SHSMRYFYTAMSRPGRGEPRFIAVGYVDDTQFVRFDSDAASPRMAPRAPWIEQEGPEYWDGETRNMKASAQTYRENLRIALRYYNQSEAGSHIIQVMYGCDVGPDGRLLRGHNQYAYDGKDYIALNEDLSSWTAADTAAQITQRKWEAAREAEQDRAYLEGLCVEWLRRYLENGKETLQRA

SEQ ID NO: 34 - protein, 181 aa, Homo sapiens
SHSMRYFYTSVSRPGRGEPRFIAVGYVDDTQFVRFDSDAASPRMAPRAPWIEQEGPEYWDGETRNMKASAQTYRENLRIALRYYNQSEAGSHIIQVMYGCDVGPDGRLLRGHDQSAYDGKDYIALNEDLSSWTAADTAAQITQRKWEAARVAEQLRAYLEGLCVEWLRRYLENGKETLQRA

SEQ ID NO: 35 - protein, 362 aa, Homo sapiens [sequence omitted]

SEQ ID NO: 36 - protein, 181 aa, Homo sapiens
SHSMRYFYTAMSRPGRGEPRFIAVGYVDDTQFVRFDSDAASPRMAPRAPWIEQEGPEYWDGETRNMKASAQTYRESLRNLRGYYNQSEAGSHIIQVMYGCDVGPDGRLLRGHNQYAYDGKDYIALNEDLSSWTAADTAAQITQRKWEAARVAEQRRAYLEGLCVEWLRRYLENGKETLQRA

SEQ ID NO: 37 - protein, 181 aa, Homo sapiens
SHSMRYFYTAMSRPGRGEPRFIAVGYVDDTQFVRFDSDAASPRMAPRAPWIEQEGPEYWDGETRNMKASAQTYRENLRIALRYYNQSEAGSHIIQVMYGCDVGPDGRLLRGHDQSAYDGKDYIALNEDLRSWTAADTAAQITQRKWEAAREAEQRRAYLEGECVEWLRRYLENGKETLQRA

SEQ ID NO: 38 - protein, 181 aa, Homo sapiens
SHSMRYFYTAMSRPGRGEPRFIAVGYVDDTQFVRFDSDAASPRMAPRAPWIEQEGPEYWDGETRNMKASAQTYRENLRIALRYYNQSEAGSHIIQVMYGCDVGPDGRLLRGHDQSAYDGKDYIALNEDLSSWTAADTAAQITQRKWEAARVAEQLRAYLEGLCVEWLRRHLENGKETLQRA

SEQ ID NO: 39 - protein, 181 aa, Homo sapiens; identical to SEQ ID NO: 38

SEQ ID NO: 40 - protein, 181 aa, Homo sapiens
SHSMRYFYTAMSRPGRGEPRFIAVGYVDDTQFVRFDSDAASPRMAPRAPWIEQEGPEYWDGETRNVKASAQTYRENLRIALRYYNQSEAGSHIIQVMYGCDVGPDGRLLRGHDQSAYDGKDYIALNEDLSSWTAADTAAQITQRKWEAARVAEQLRAYLEGLCVEWLRRYLENGKETLQRA

SEQ ID NO: 41 - protein, 181 aa, Homo sapiens
SHSMRYFYTAMSRPGRGEPRFIAVGYVDDTQFVRFDSDAASPRMEPRAPWIEQEGPEYWDGETRNMKASAQTYRENLRIALRYYNQSEAGSHIIQVMYGCDVGPDGRLLRGHDQSAYDGKDYIALNEDLSSWTAADTAAQITQRKWEAARVAEQLRAYLEGLCVEWLRRYLENGKETLQRA

SEQ ID NO: 42 - protein, 181 aa, Homo sapiens
SHSMRYFYTAMSRPGRGEPRFIAVGYVDDTQFVRFDSDAASPRMAPRAPWIEQEGPEYWDGETRNMKASAQTYRENLRIALRYYNQSEAGSHIIQVMYGCDVGPDGRLLRGHNQYAYDGKDYIDLNEDLSSWTAADTAAQITQRKWEAARVAEQLRAYLEGLCVEWLRRYLENGKETLQRA

SEQ ID NO: 43 - protein, 181 aa, Homo sapiens
SHSMRYFYTAMSRPGRGEPRFIAVGYVDDTQFVRFDSDAASPRMAPRAPWIEQEGPEYWDGETRNMKASAQTYRENLRIALRYYNQSEAGSHIIQVMYGCDVGPDGRLLRGHDQSAYDGKDYIALNEDLSSWTAAYTAAQITQRKWEAARVAEQLRAYLEGLCVEWLRRYLENGKETLQRA

SEQ ID NO: 44 - protein, 181 aa, Homo sapiens
SHSMRYFYTAMSRPGRGEPRFIAVGYVDDTQFVRFDSDAASPRMAPRAPWIEQEGPEYWDGETRNMKASAQTYRENLRIALRYYNQSEAGSHIIQVMYGCDVGPDGRLLRGHDQSAYDGKDYIALNEDLSSWTAADTAAQITQRKWEAARVAEQRRAYLEGLCVEWLRRYLENGKETLQRA

SEQ ID NO: 45 - protein, 181 aa, Homo sapiens
SHSMRYFYTAMSRPGRGEPRFIAVGYVDDTQFVRFDSDAASPRMAPRAPWIEQEGPEYWDGKTRNMKASAQTYRENLRIALRYYNQSEAGSHIIQVMYGCDVGPDGRLLRGHDQSAYDGKDYIALNEDLSSWTAADTAAQITQRKWEAARVAEQLRAYLEGLCVEWLRRYLENGKETLQRA

SEQ ID NO: 46 - protein, 181 aa, Homo sapiens
SHSMRYFYTAMSRPGRGEPRFIAVGYVDDTQFVRFDSDAASPRMAPRAPWIEQEGPEYWDGETRNMKASAQTYRENLRIALRYYNQSEAGSHVIQVMYGCDVGPDGRLLRGHDQSAYDGKDYIALNEDLSSWTAADTAAQITQRKWEAARVAEQLRAYLEGLCVEWLRRYLENGKETLQRA

SEQ ID NO: 47 - protein, 181 aa, Homo sapiens
SHSMRYFYTAMSRPGRGEPRFIAVGYVDDTQFVRFDSDAASPRMAPRAPWIEQEGPEYWDGETRNMKASAQTYRENLRIALRYYNQSEAGSHIIQVMYGCDVGPDGRLLRGHDQSAYDGKDYIALNEDLSSWTAADTAAQITQRKWEAAREAEQLRAYLEGLCVEWLRRYLENGKETLQRA

SEQ ID NO: 48 - protein, 181 aa, Homo sapiens
SHSMRYFYTAMSRPGRGESRFIAVGYVDDTQFVRFDSDAASPRMAPRAPWIEQEGPEYWDGETRNMKASAQTYRENLRIALRYYNQSEAGSHIIQVMYGCDVGPDGRLLRGHDQSAYDGKDYIALNEDLSSWTAADTAAQITQRKWEAARVAEQLRAYLEGLCVEWLRRYLENGKETLQRA

SEQ ID NO: 49 - protein, 181 aa, Homo sapiens
SHSMRYFYTAMSRPGRGEPRFIAVGYVDDTQFVRFDSDAASPRMAPRAPWIEQEGPEYWDGETRNMKASAQTYRENLRIALRYYNQSEAGSHIIQVMYGCDVGPDGRLLRGHDQSAYDGKDYIALNEDLSSWTAADTAAQITQRKWEAARVAEQDRAYLEGLCVEWLRRYLENGKETLQRA

SEQ ID NO: 50 - protein, 181 aa, Homo sapiens
SHSMRYFYTAMSRPGRGEPRFIAVGYVDDTQFVRFDSDAASPRMAPRAPWIEQEGPEYWDGETRNMKASAQTYRENLRIALRYYNQSEAGSHIIQVMYGCDVGPDGRLLRGHDQSAYDGKDYIALNEDLSSWTAADTAAQITQRKWEAARVAEQLRAYLEGECVEWLRRYLENGKETLQRA

SEQ ID NO: 51 - protein, 181 aa, Homo sapiens
SHSMRYFYTAMSRPGRGEPRFIAVGYVDDTQFVRFDSDAASPRMAPRAPWIEQEGPEYWDGETRNMKASAQTYRENLRIALRYYNQSEAGSHIIQVMYGCDVGPDGRLLRGHDQSAYDGKDYIALNEDLSSWTAADTAAQITQRKWEAARVAEQLRAYLEGTCVEWLRRYLENGKETLQRA

SEQ ID NO: 52 - protein, 181 aa, Homo sapiens
SHSMRYFYTAMSRPGRGEPRFIAVGYVDDTQFVRFDSDAASPRMAPRAPWIEQEGPEYWDGETRNMKASAQTYRENLRIALRYYNQSEAGSHIIQVMYGCDVGPDGRLLRGHDQSAYDGKDYIALNEDLSSWTAADTAAQITQRKWEAARVAEHLRAYLEGLCVEWLRRYLENGKETLQRA

SEQ ID NO: 53 - protein, 115 aa, Homo sapiens
  misc_feature (115)..(115): Xaa can be any naturally occurring amino acid
SHSMRYFYTAMSRPGRGEPRFIAVGYVDDTQFVRFDSDAASPRMAPRAPWIEQEGPEYWDGETRNMKASAQTYRENLRIALRYYNQSEAGSHIIQVMYGCDVGPDGRLLRGHNQX

SEQ ID NO: 54 - protein, 362 aa, Homo sapiens [sequence omitted]

SEQ ID NO: 55 - protein, 181 aa, Homo sapiens
SHSMRYFYTAMSRPGRGEPRFIAVGYVDDTQFVRFDSDAASPRMAPRAPWIEQEGPEYWDGETRNMKASAQTYRENLRIALRYYNQSEAGSHIIQVMYGCDVGPDGRLLRGHDQSAYDGKDYIALNEDLSSWTAADTAAQITQRKWEAARAAEQRRAYLEGLCVEWLRRYLENGKETLQRA

SEQ ID NO: 56 - protein, 181 aa, Homo sapiens
SHSMRYFYTAMSRPGRGEPRFIAVGYVDDTQFVRFDSDAASPRMAPRAPWIEQEGPEYWDGETRNMKASAQTYRENLRIALRYYNQSEAGSHIIQVMYGCDVGPDGRLLRGHDQSAYDGKDYIALNEDLRSWTAADTAAQITQRKWEAARVAEQLRAYLEGLCVEWLRRYLENGKETLQRA

SEQ ID NO: 57 - protein, 181 aa, Homo sapiens
SHSMRYFYTAMSRPGRGEPRFIAVGYVDDTQFVRFDSDAASPRMAPRAPWIEQEGPEYWDGETRNMKASAQTYRENLRIALRYYNQSEAGSHIIQVMYGCDVGPDGRLLRGYHQDAYDGKDYIALNEDLSSWTAADTAAQITQRKWEAARVAEQLRAYLEGLCVEWLRRYLENGKETLQRA

SEQ ID NO: 58 - protein, 108 aa, Homo sapiens
SHSMRYFYTAMSRPGRGEPRFIAVGYVDDTQFVRFDSDAASPRMAPRAPWIEQEGPEYWDGETRNMKASAQTYRENLRIALRYYNQSEAGSHIIQVMYGCDVGPDERL

SEQ ID NO: 59 - protein, 73 aa, Homo sapiens
LRGHDQSAYDGKDYIALNEDLSSWTAADTAAQITQRKWEAARVAEQLRAYLEGLCVEWLRRYLENGKETLQRA

SEQ ID NO: 60 - protein, 181 aa, Homo sapiens
SHSMRYFYTAMSRPGRGEPRFIAVGYVDDTQFVRFDSDAASRRMAPRAPWIEQEGPEYWDGETRNMKASAQTYRENLRIALRYYNQSEAGSHIIQVMYGCDVGPDGRLLRGHDQSAYDGKDYIALNEDLSSWTAADTAAQITQRKWEAARVAEQLRAYLEGLCVEWLRRYLENGKETLQRA

SEQ ID NO: 61 - protein, 181 aa, Homo sapiens
SHSMRYFYTAMSRPGRGEPRFIAVGYVDDTQFVRFDSDAASPRMAPRAPWIEQEGPKYWDGETRNMKASAQTYRENLRIALRYYNQSEAGSHIIQVMYGCDVGPDGRLLRGHDQSAYDGKDYIALNEDLSSWTAADTAAQITQRKWEAARVAEQLRAYLEGLCVEWLRRYLENGKETLQRA

SEQ ID NO: 62 - protein, 181 aa, Homo sapiens
SHSMRYFYTAMSRPGRGEPRFIAVGYVDDTQFVRFDSDAASPRMAPRAPWIEQEGPEYWDGETRHMKASAQTYRENLRIALRYYNQSEAGSHIIQVMYGCDVGPDGRLLRGHDQSAYDGKDYIALNEDLSSWTAADTAAQITQRKWEAARVAEQLRAYLEGLCVEWLRRYLENGKETLQRA

SEQ ID NO: 63 - protein, 273 aa, Homo sapiens
SHSMRYFYTAMSRPGRGEPRFIAVGYVDDTQFVRFDSDAASPRMAPRAPWIEQEGPEYWDGETRNMKASAQTYRENLRIALRYYNQSEAGSHIIQVMYGCDVGPDGRLLRGHDQSAYDGKDYIALNEDLSSWTAADTAAQITQRKWEAARVAEQLRAYLEGLCVEWLRRYLENGKETLQRADPPKTHVTHHPISDHEATLRCWALGFYPAEITLTWQRDGEDQTQDTELVETRPAGDRTFQKWAAVVVPSGEEQRYTCHVQHEGLPKHLTLRW

SEQ ID NO: 64 - protein, 181 aa, Homo sapiens
SHSMRYFYTAMSRPGRGEPRFIAVGYVDDTQFVRFDSDAASPRMAPRAPWIEQEGPEYWDGETRNMKASAQTYRETLRIALRYYNQSEAGSHIIQVMYGCDVGPDGRLLRGHDQSAYDGKDYIALNEDLSSWTAADTAAQITQRKWEAARVAEQLRAYLEGLCVEWLRRYLENGKETLQRA

SEQ ID NO: 65 - protein, 181 aa, Homo sapiens
SHSMRYFHTAMSRPGRGEPRFIAVGYVDDTQFVRFDSDAASPRMAPRAPWIEQEGPEYWDGETRNMKASAQTYRENLRIALRYYNQSEAGSHIIQVMYGCDVGPDGRLLRGHNQYAYDGKDYIALNEDLSSWTAADTAAQITQRKWEAARVAEQLRAYLEGLCVEWLRRYLENGKETLQRA

SEQ ID NO: 66 - protein, 181 aa, Homo sapiens
SHSMRYFYTAMSRPGRGEPRFIAVGYVDDTQFVRFDSDAASPRMAPRAPWIEQEGPEYWDGETRNMKASAQTYRENLRIALRYYNQSEAGSHNIQVMYGCDVGPDGRLLRGHDQSAYDGKDYIALNEDLSSWTAADTAAQITQRKWEAARVAEQLRAYLEGLCVEWLRRYLENGKETLQRA

SEQ ID NO: 67 - protein, 181 aa, Homo sapiens
SHSMRYFYTAMSRPGRGEPRFIAVGYVDDTQFVRFDSDAASPRMAPRAPWIEQEGPEYWDGETRNMKASAQTYRENLRIALRYYNQSEAGSHIIQVMYGCDVGPDGRLLRGYDQSAYDGKDYIALNEDLSSWTAADTAAQITQRKWEAARVAEQLRAYLEGLCVEWLRRYLENGKETLQRA

SEQ ID NO: 68 - protein, 181 aa, Homo sapiens
SHSMRYFYTAMSRPGRGEPRFIAVGYVDDTQFVRFDSDAASPRMAPRAPWIEQEGPEYWDGETRNMKASAQTYRENLRIALRYYNQSEAGSHIIQVMYGCDVGPDGRLLRGHNQYAYDGKDYIALNEDLSSWTAADTAAQITQRKWEEARVAEQRRAYLEGLCVEWLRRYLENGKETLQRA

SEQ ID NO: 69 - protein, 181 aa, Homo sapiens
SHSMRYFYTAMSRPGRGEPRFIAVGYVDDTQFVRFDSDAASPRMAPRAPWIEQEGPEYWDGETRNMKASAQTYRENLRIALRYYNQSEAGSHIIQVMYGCDVGPDGRLLRGHDQSAYDGKDYIALNEDLSSWTAADTAAQITQRKWEAARVAEQLRAYLEGPCVEWLRRYLENGKETLQRA

SEQ ID NO: 70 - protein, 181 aa, Homo sapiens
SHSMRYFYTAMSRPGLGEPRFIAVGYVDDTQFVRFDSDAASPRMAPRAPWIEQEGPEYWDGETRNMKASAQTYRENLRIALRYYNQSEAGSHIIQVMYGCDVGPDGRLLRGHDQSAYDGKDYIALNEDLSSWTAADTAAQITQRKWEAARVAEQLRAYLEGLCVEWLRRYLENGKETLQRA

SEQ ID NO: 71 - protein, 181 aa, Homo sapiens
SHSMRYFYTAMSRPGRGEPRFIAVGYVDDTQFVRFDSDATSPRKEPRAPWIEQEGPEYWDGETRNMKASAQTYRENLRIALRYYNQSEAGSHIIQVMYGCDVGPDGRLLRGHDQSAYDGKDYIALNEDLSSWTAADTAAQITQRKWEAARVAEQLRAYLEGLCVEWLRRYLENGKETLQRA

SEQ ID NO: 72 - protein, 181 aa, Homo sapiens
SHSMRYFYTAMSRPGRGEPRFIAVGYVDDTQFVRFDSDAASPRMAPRAPWIEQEGPEYWDGETRNMKASAQTYRENLRIALRYYNQSEAGSHIIQVMYGCDVGPDGRLLRGHNQYAYDGKDYIALNEDLSSWTAADTAAQITQRKWEAACVAEQLRAYLEGLCVEWLRRYLENGKETLQRA

SEQ ID NO: 73 - protein, 181 aa, Homo sapiens
SHSMRYFYTAMSRPGRGEPRFIAVGYVDDTQFVRFDSDAASPRMAPRAPWIEQEGPEYWDGETRNMKASAQTYRENLRIALRYYNQSEAGSHIIQVMYGCDVGPDGRLLRGHDQSAYDGKDYIALNEDLSCWTAADTAAQITQRKWEAARVAEQLRAYLEGLCVEWLRRYLENGKETLQRA

SEQ ID NO: 74 - protein, 273 aa, Homo sapiens
SHSMRYFYTAMSRPGRGEPRFIAVGYVDDTQFVRFDSDAASPRMAPRAPWIEQEGPEYWDGETRNMKASAQTYRENLRIALRYYNQSEAGSHIIQVMYGCDVGPDGPLLRGHDQSAYDGKDYIALNEDLSSWTAADTAAQITQRKWEAARVAEQLRAYLEGLCVEWLRRYLENGKETLQRADPPKTHVTHHPISDHEATLRCWALGFYPAEITLTWQRDGEDQTQDTELVETRPAGDRTFQKWAAVVVPSGEEQRYTCHVQHEGLPKPLTLRW

SEQ ID NO: 75 - protein, 181 aa, Homo sapiens
SHSMRYFDTAMSRPGRGEPRFIAVGYVDDTQFVRFDSDAASPRMAPRAPWIEQEGPEYWDGETRNMKASAQTYRENLRIALRYYNQSEAGSHIIQVMYGCDVGPDGRLLRGHDQSAYDGKDYIALNEDLSSWTAADTAAQITQRKWEAARVAEQLRAYLEGLCVEWLRRYLENGKETLQRA

SEQ ID NO: 76 - protein, 181 aa, Homo sapiens
SHSMRYFYTAMSRPGRGEPRFIAVGYVDDTQFVRFDSDAASPRMAPRAPWIEQEGPEYWDGETRNMKASAQTYRENLRIALRYYNQSEAGSHIIQVMYGCDVGPDGRLLRGHDQSAYDGKDYIALNEDLSSWTAADTAAQITQGKWEAARVAEQLRAYLEGLCVEWLRRYLENGKETLQRA

SEQ ID NO: 77 - protein, 181 aa, Homo sapiens
SHSMRYFHTAMSRPGRGEPRFITVGYVDDTLFVRFDSDATSPRKEPRAPWIEQEGPEYWDGETRNMKASAQTYRENLRIALRYYNQSEAGSHIIQVMYGCDVGPDGRLLRGHDQSAYDGKDYIALNEDLSSWTAADTAAQITQRKWEAARVAEQLRAYLEGLCVEWLRRYLENGKETLQRA

SEQ ID NO: 78 - protein, 181 aa, Homo sapiens
SHSMRYFYTAMSRPGRGEPRFIAVGYVDDTQFVRFDSDAASPRMAPRAPWIEQEGPEYWDGETRNMKASAQTYRENLRIALRYYNQSEAGSHIIQVMYGCDVGPDGRLLRGHDQSAYDGKDYIALNEDLSSWTAADTAAQITQRKWEAARVAEQLRASLEGLCVEWLRRYLENGKETLQRA

SEQ ID NO: 79 - protein, 181 aa, Homo sapiens
SHSMRYFYTAMSRPGRGEPRFIAVGYVDDTQFVRFDSDAASPRMAPRAPWIEQEGPEYWDGETRNMKASAQTYRENLRIALRYYNQSEAGSHIIQVMYGCDVGPDGRLLRGHDQSTYDGKDYIALNEDLSSWTAADTAAQITQRKWEAARVAEQLRAYLEGLCVEWLRRYLENGKETLQRA

SEQ ID NO: 80 - protein, 181 aa, Homo sapiens
SHSMRYFYTAMSRPGRGEPRFIAVGYVDDTQFVRFDSDAASPRMAPRAPWIEQEGPEYWDGETRNMKASAQTYRENLRIALRYYNQSEAGSHIIQVMYGCDVGPDGRLLRGHDQSAYDGKDYIALNEDLSSWTAADKAAQITQRKWEAARVAEQLRAYLEGLCVEWLRRYLENGKETLQRA

SEQ ID NO: 81 - protein, 273 aa, Homo sapiens
SHSMRYFYTAMSRPGRGEPRFIAVGYVDDTQFVRFDSDAASPRMAPRAPWIEQEGPEYWDGETRNMKASAQTYRENLRIALRYYNQSEAGSHIIQVMYGCDVGPDGRLLRGHDQSAYDGKDYIALNEDLSSWTAADTAAQITQRKWEAARVAEQLRAYLEGLCVEWLRRYLENGKETLQRADPPKTHVTHHPISDHEATLRCWALGFYPAEITLTWQRDGEDQTQDTKLVETRPAGDRTFQKWAAVVVPSGEEQRYTCHVQHEGLPKPLTLRW

SEQ ID NO: 82 - protein, 181 aa, Homo sapiens
SHSMRYFYTAMSRPGRGEPRFIAVGYVDDTQFVRFDSDAASPRMAHRAPWIEQEGPEYWDGETRNMKASAQTYRENLRIALRYYNQSEAGSHIIQVMYGCDVGPDGRLLRGHDQSAYDGKDYIALNEDLSSWTAADTAAQITQRKWEAARVAEQLRAYLEGLCVEWLRRYLENGKETLQRA

SEQ ID NO: 83 - protein, 273 aa, Homo sapiens
SHSMRYFYTAMSRPGRGEPRFIAVGYVDDTQFVRFDSDAASPRMAPRAPWIEQEGPEYWDGETRNMKASAQTYRENLRIALRYYNQSEAGSHIIQVMYGCDVGPDGRLLRGHNQYAYDGKDYIALNEDLSSWTAADTAAQITQRKWEAAREAEQLRAYLEGLCVEWLRRYLENGKETLQRADPPKTHVTHHPISDHEATLRCWALGFYPAEITLTWQRDGEDQTQDTELVETRPAGDRTFQKWAAVVVPSGEEQRYTCHVQHEGLPKPLTLRW

SEQ ID NO: 84 - protein, 181 aa, Homo sapiens
SHSMRYFYTAMSRPGRGEPRFISVGYVDDTQFVRFDSDAASPRMAPRAPWIEQEGPEYWDGETRNMKASAQTYRENLRIALRYYNQSEAGSHIIQVMYGCDVGPDGRLLRGHDQSAYDGKDYIALNEDLSSWTAADTAAQITQRKWEAARVAEQLRAYLEGLCVEWLRRYLENGKETLQRA

SEQ ID NO: 85 - protein, 273 aa, Homo sapiens
SHSMRYFYTAMSRPGRGEPRFIAVGYVDDTQFVRFDSDAASPRMAPRAPWIEQEGPEYWDGETRNMKASAQTYRENLRIALRYYNQSEAGSHIIQVMYGCDVGPDGRLLRGHDQSAYDGKDYIALNEDLSSWTAADTAAQISQRKLEAARVAEQLRAYLEGLCVEWLRRYLENGKETLQRADPPKTHVTHHPISDHEATLRCWALGFYPAEITLTWQRDGEDQTQDTELVETRPAGDRTFQKWAAVVVPSGEEQRYTCHVQHEGLPKPLTLRW

SEQ ID NO: 86 - protein, 181 aa, Homo sapiens
SHSMRYFYTAMSRPGRGEPRFIAVGYVDDTQFVRFDSDAASPRMAPRAPWIEQEGPEYWDGETRNMKASAQTYRESLRIALRYYNQSEAGSHIIQVMYGCDVGPDGRLLRGHDQSAYDGKDYIALNEDLSSWTAADTAAQITQRKWEAARVAEQLRAYLEGLCVEWLRRYLENGKETLQRA

SEQ ID NO: 87 - protein, 181 aa, Homo sapiens
SHSMRYFYTAMSRPGRGEPRFIAVGYVDDTQFVRFDSDAASPRMAPRAPWIEQEGPEYWDGETRNMKASAQTYRENLRIALRYYNQSEAGSHIIQVMYGCDVGPDGRLLRGHDQSAYDGKDYIALNEDLSSWTAADTAAQITQRKWEAARVAEQLRAYLGGLCVEWLRRYLENGKETLQRA

SEQ ID NO: 88 - protein, 181 aa, Homo sapiens
SHSMRYFYTAMSRPGRGEPRFIAVGYVDDTQFVRFDSDAASPRMAPRAPWIEQEGPEYWDGEKRNMKASAQTYRENLRIALRYYNQSEAGSHIIQVMYGCDVGPDGRLLRGHDQSAYDGKDYIALNEDLSSWTAADTAAQITQRKWEAARVAEQLRAYLEGLCVEWLRRYLENGKETLQRA

SEQ ID NO: 89 - protein, 181 aa, Homo sapiens
SHSMRYFYTAMSRPGRGEPRFIAVGYVDDTQFVRFDSDAASPRMAPRAPWIEQEGPEYWDGETRNMKASAQTYRENLRIALRYYNQSEAGSHIIQVMYGCDVGPDGRLLRGHNQYAYDGKDYIALNEDLSSWTAADTAAQITQRKWEAAREAEQRRAYLEGLCVEWLRRYLENGKETLQRA

SEQ ID NO: 90 - protein, 181 aa, Homo sapiens
SHSMRYFYTAMSRPGRGEPRFIAVGYVDDTQFVRFDSDAASPRMAPRAPWIEQEGPEYWDGETRNMKASAQTYRENLRIALRYYNQSEAGSHIIQVMYGCDVGPDGRLLRGHDQSAYDGKDYIALNEDLSSWTAADTAAQITQRKWEAACVAEQLRAYLEGLCVEWLRRYLENGKETLQRA

SEQ ID NO: 91 - protein, 181 aa, Homo sapiens
SHSMRYFYTAMSRPGRGEPRFIAVGYVDDTQFVRFDSDAASPRMAPRAPWIEQEGPEYWDGETRNMKASAQTYRENLRIALRYYNQSEAGSHIIQVMYGCDVGPDGRLLRGHDQSAYDGKDYIALNEDLSSWTAADTAAQITQRKWEAVRVAEQLRAYLEGLCVEWLRRYLENGKETLQRA

SEQ ID NO: 92 - protein, 181 aa, Homo sapiens
SHSMRYFYTAMSRPGRGEPRFIAVGYVDDTQFVRFDSDAASPRMAPRAPWIEQEGPEYWDGETRNMKASAQTYRENLRIALRYYNQSEAGSHIIQVMYGCDVGPDGRLLRGHNQYAYDGKDYIALNEDLSSRTAADTAAQITQRKWEAARVAEQLRAYLEGLCVEWLRRYLENGKETLQRA

SEQ ID NO: 93 - protein, 181 aa, Homo sapiens
SHSMRYFYTAMSRPGRGEPRFIAVGYVDDTQFVRFDSDAASPRMAPRAPWIEQEGPEYWDGETRNMKASAQTYRENLRIALRYYNQSEAGSHIIQVMYGCDLGPDGRLLRGHDQSAYDGKDYIALNEDLSSWTAADTAAQITQRKWEAARVAEQLRAYLEGLCVEWLRRYLENGKETLQRA

SEQ ID NO: 94 - protein, 181 aa, Homo sapiens; identical to SEQ ID NO: 93

SEQ ID NO: 95 - protein, 181 aa, Homo sapiens
SHSMRYFYTAMSRPGRGEPRFIAVGYVDDTQFVRFDSDAASPRMAPRAPWIEQEGPEYWDGETRNMKASAQTYRENLRIALRYYNQSEAGSHIIQVMYGCDVGPDGRLLRGHDQSAYDGKDYIALNEDLSSWTAADTAAQITKRKWEAARVAEQLRAYLEGLCVEWLRRYLENGKETLQRA

SEQ ID NO: 96 - protein, 181 aa, Homo sapiens
SHSMRYFYTAMSRPGRGEPRFITVGYVDDTLFVRFDSDATSPRKEPRAPWIEQEGPEYWDGETRNMKASAQTYRENLRIALRYYNQSEAGSHIIQVMYGCDVGPDGRLLRGHDQSAYDGKDYIALNEDLSSWTAADTAAQITQRKWEAARVAEQLRAYLEGLCVEWLRRYLENGKETLQRA

SEQ ID NO: 97 - protein, 181 aa, Homo sapiens
SHSMRYFYTAMSRPGRGEPRFIAVGYVDDTQFVRFDSDAASPRMAPRAPWIEQEGPEYWDGETRNMKASAQTYRENLRIALRYYNQSEAGSHIIQVMYGCDVGPDGRLLRGHNQYAYDGKDYIALNEDLSSWTAADTAAQITQRKWEAARVAEQLRAYLEGLCVECLRRYLENGKETLQRA

SEQ ID NO: 98 - protein, 273 aa, Homo sapiens
SHSMRYFYTAMSRPGRGEPRFITVGYVDDTQFVRFDSDATSPRMAPRAPWIEQEGPEYWDGETRNMKASAQTYRENLRIALRYYNQSEAGSHIIQVMYGCDVGPDGRLLRGHDQSAYDGKDYIALNEDLSSWTAADTAAQITQRKWEAARVAEQLRAYLEGLCVEWLRRYLENGKETLQRADPPKTHVTHHPISDHEATLRCWALGFYPAEITLTWQRDGEDQTQDTELVETRPAGDRTFQKWAAVVVPSGEEQRYTCHVQHEGLPKPLTLRW

SEQ ID NO: 99 - protein, 181 aa, Homo sapiens
SHSMRYFYTAMSRPGRGEPRFIAVGYVDDTQFVRFDSDAASPRMAPRAPWIEQEGPEYWDGETRNMKASAQTYRENLRIALRYYNQSEAGSHIIQVMYGCDVGPDGRLLRGHDQSAYDGKDYIALNEDLSSWTAADTAAQITQRKWEAARVADQLRAYLEGLCVEWLRRYLENGKETLQRA

SEQ ID NO: 100 - protein, 181 aa, Homo sapiens
SHSMRYFHTAMSRPGRGEPRFIAVGYVDDTQFVRFDSDAASPRMAPRAPWIEQEGPEYWDGETRNMKASAQTYRENLRIALRYYNQSEAGSHIIQVMYGCDVGPDGRLLRGHDQSAYDGKDYIALNEDLSSWTAADTAAQITQRKWEAARVAEQLRAYLEGLCVEWLRRYLENGKETLQRA

SEQ ID NO: 101 - protein, 181 aa, Homo sapiens
SHSMRYFYTAMSRPGRGEPRFIAVGYVDDTQFVRFDSDAASPRMAPRAPWIEQEGPEYWDGETRNMKASAQTYRENLRIALRYYNQSEAGSYIIQVMYGCDVGPDGRLLRGHDQSAYDGKDYIALNEDLSSWTAADTAAQITQRKWEAARVAEQLRAYLEGLCVEWLRRYLENGKETLQRA

SEQ ID NO: 102 - protein, 181 aa, Homo sapiens
SHSMRYFYTAMSRPGRGEPRFIAVGYVDDTQFVRFDSDAASPRMAPRATWIEQEGPEYWDGETRNMKASAQTYRENLRIALRYYNQSEAGSHIIQVMYGCDVGPDGRLLRGHDQSAYDGKDYIALNEDLSSWTAADTAAQITQRKWEAARVAEQLRAYLEGLCVEWLRRYLENGKETLQRA

SEQ ID NO: 103 - protein, 181 aa, Homo sapiens
SHSMRYFYTAMSRPGRGEPRFIAVGYVDDTQFVRFDSDAASPRMAPRAPWIEQEGPEYWDGETRNMKASAQTYRENLRIALRYYNQSEAGSHIIQVMYGCDVGPDGRLLRGHDQFAYDGKDYIALNEDLSSWTAADTAAQITQRKWEAARVAEQLRAYLEGLCVEWLRRYLENGKETLQRA

SEQ ID NO: 104 - protein, 181 aa, Homo sapiens
SHSMRYFYTAMSRPGRGEPRFIAVGYVDDTQFVRFDSDAASPRMAPRAPWIEQEGPEYWDGETRNMKASAQTYRENLRIALRYYNQSEAGSHIIQVMYGCDVGPDGLLLRGHDQSAYDGKDYIALNEDLSSWTAADTAAQITQRKWEAARVAEQLRAYLEGLCVEWLRRYLENGKETLQRA

SEQ ID NO: 105 - protein, 181 aa, Homo sapiens
SHSMRYFYTAMSRPGRGEPRFIAVGYVDDTQFVRFDSDAASPRMAPWAPWIEQEGPEYWDGETRNMKASAQTYRENLRIALRYYNQSEAGSHIIQVMYGCDVGPDGRLLRGHDQSAYDGKDYIALNEDLSSWTAADTAAQITQRKWEAARVAEQLRAYLEGLCVEWLRRYLENGKETLQRA

SEQ ID NO: 106 - protein, 296 aa, Homo sapiens
  misc_feature (296)..(296): Xaa can be any naturally occurring amino acid
MRVTAPRTVLLLLWGAVALTETWAGSHSMRYFYTAMSRPGRGEPRFIAVGYVDDTQFVRFDSDAASPRMAPRAPWIEQEGPEYWDGETRNMKASAQTYRENLRIALRYYNQSEAGSHIIQVMYGCDVGPDGRLLRGHDQSAYDGKDYIALNEDLSSWTAADTAAQITQRKWEAARVAEQLRAYLEGLCVEWLRRYLENGKETLQRADPPKTHVTHHPISDHEATLRCWALGFYPAEITLTWQRDGEDQTQDTELVETRPAGDRTFQKWAAVVVPSGEEQRYTCHVQHEGLPNPSPX

SEQ ID NO: 107 - protein, 181 aa, Homo sapiens
SHSMRYFYTAMSRPGRGEPRFISVGYVDDTQFVRFDSDAASPRMAPRAPWIEQEGPEYWDGETRNMKASAQTYRENLRIALRYYNQSEAGSHIIQVMYGCDVGPDGRLLRGHNQYAYDGKDYIALNEDLSSWTAADTAAQITQRKWEAARVAEQLRAYLEGLCVEWLRRYLENGKETLQRA

SEQ ID NO: 108 - protein, 181 aa, Homo sapiens
SHSMRYFYTAMSRPGRGEPRFIAVGYVDDTQFVRFDSDAASPRMAPRAPWIEQEGPEYWEGETRNMKASAQTYRENLRIALRYYNQSEAGSHIIQVMYGCDVGPDGRLLRGHDQSAYDGKDYIALNEDLSSWTAADTAAQITQRKWEAARVAEQLRAYLEGLCVEWLRRYLENGKETLQRA

SEQ ID NO: 109 - protein, 362 aa, Homo sapiens [sequence omitted]

SEQ ID NO: 110 - protein, 15 aa, Artificial Sequence
  Linker Sequence connecting HLA-B57 polypeptide with Fc domain
GGGGSGGGGSGGGGS